European Patent Application EP 4 134 960 A1, published February 15, 2023. Title: DETERMINING A NUCLEIC ACID SEQUENCE IMBALANCE. Applicant: The Chinese University of Hong Kong. Application EP, filed July 23, 2008. The sequence listing filed with the application follows.

SEQUENCE LISTING (58 sequences)

SEQ ID NO: 1 - DNA, 27 bp, synthetic construct
  source 1..27: mol_type = other DNA
  misc_feature 1..27: note = synthetic real-time PCR and digital RNA-SNP analysis PLAC4 gene-specific reverse transcription primer
agtatatagaaccatgtttaggccaga

SEQ ID NO: 2 - DNA, 21 bp, synthetic construct
  source 1..21: mol_type = other DNA
  misc_structure 1..21: note = synthetic real-time PCR PLAC4 primer
ccgctagggtgtcttttaagc

SEQ ID NO: 3 - DNA, 25 bp, synthetic construct
  source 1..25: mol_type = other DNA
  misc_feature 1..25: note = synthetic real-time PCR PLAC4 primer
gtgttgcaatacaaaatgagtttct

SEQ ID NO: 4 - DNA, 14 bp, synthetic construct
  source 1..14: mol_type = other DNA
  modified_base 1: mod_base = OTHER; note = a modified by 6-carboxyfluorescein (FAM)
  modified_base 14: mod_base = OTHER; note = c modified by minor groove binding non-fluorescent quencher (MGBNFQ)
  misc_feature 1..14: note = synthetic real-time PCR PLAC4 fluorescent probe
attggagcaaattc

SEQ ID NO: 5 - DNA, 104 bp, synthetic construct
  source 1..104: mol_type = other DNA
  misc_feature 1..104: note = single-stranded synthetic DNA oligonucleotide amplicon
cgccgctagggtgtcttttaagctattggagcaaattcaaatttggcttaaagaaaaagaaactcattttgtattgcaacaccaggagtatcccaagggactcg

SEQ ID NO: 6 - DNA, 22 bp, synthetic construct
  source 1..22: mol_type = other DNA
  misc_feature 1..22: note = synthetic digital RNA-SNP analysis non-intron spanning forward primer
tttgtattgcaacaccatttgg

SEQ ID NO: 7 - DNA, 15 bp, synthetic construct
  source 1..15: mol_type = other DNA
  modified_base 1: mod_base = OTHER; note = t modified by 6-carboxyfluorescein (FAM)
  modified_base 15: mod_base = OTHER; note = g modified by minor groove binding non-fluorescent quencher (MGBNFQ)
  misc_feature 1..15: note = synthetic allele-G-specific TaqMan probe targeting rs8130833 SNP of PLAC4
tcgtcgtctaacttg

SEQ ID NO: 8 - DNA, 17 bp, synthetic construct
  source 1..17: mol_type = other DNA
  modified_base 1: mod_base = OTHER; note = a modified by fluorescent reporter VIC
  modified_base 17: mod_base = OTHER; note = g modified by minor groove binding non-fluorescent quencher (MGBNFQ)
  misc_feature 1..17: note = synthetic allele-A-specific TaqMan probe targeting rs8130833 SNP of PLAC4
attcgtcatctaacttg

SEQ ID NO: 9 - DNA, 23 bp, synthetic construct
  source 1..23: mol_type = other DNA
  misc_feature 1..23: note = synthetic digital RCD analysis co-amplification forward primer for paralogous loci on chromosome 21 and 1
gttgttctgcaaaaaaccttcga

SEQ ID NO: 10 - DNA, 28 bp, synthetic construct
  source 1..28: mol_type = other DNA
  misc_feature 1..28: note = synthetic digital RCD analysis co-amplification reverse primer for paralogous loci on chromosome 21 and 1
cttggccagaaatacttcattaccatat

SEQ ID NO: 11 - DNA, 19 bp, synthetic construct
  source 1..19: mol_type = other DNA
  modified_base 1: mod_base = OTHER; note = t modified by 6-carboxyfluorescein (FAM)
  modified_base 19: mod_base = OTHER; note = a modified by minor groove binding non-fluorescent quencher (MGBNFQ)
  misc_feature 1..19: note = synthetic chromosome-specific TaqMan probe designed to target chromosome 21 paralog
tacctccataatgagtaaa

SEQ ID NO: 12 - DNA, 20 bp, synthetic construct
  source 1..20: mol_type = other DNA
  misc_feature 1..20: note = synthetic chromosome-specific TaqMan probe designed to target chromosome 1 paralog
  modified_base 1: mod_base = OTHER; note = c modified by fluorescent reporter VIC
  modified_base 20: mod_base = OTHER; note = a modified by minor groove binding non-fluorescent quencher (MGBNFQ)
cgtacctctgtaatgtgtaa

SEQ ID NO: 13 - DNA, 27 bp, synthetic construct
  source 1..27: mol_type = other DNA
  misc_feature 1..27: note = synthetic digital PCR PLAC4 gene-specific reverse transcription primer
agtatatagaaccatgtttaggccaga

SEQ ID NO: 14 - DNA, 22 bp, synthetic construct
  source 1..22: mol_type = other DNA
  misc_feature 1..22: note = synthetic digital PCR amplification forward primer for rs8130833 SNP region of PLAC4 gene
tttgtattgcaacaccatttgg

SEQ ID NO: 15 - DNA, 15 bp, synthetic construct
  source 1..15: mol_type = other DNA
  modified_base 1: mod_base = OTHER; note = t modified by 6-carboxyfluorescein (FAM)
  modified_base 15: mod_base = OTHER; note = g modified by minor groove binding non-fluorescent quencher (MGBNFQ)
  misc_feature 1..15: note = synthetic allele-G-specific TaqMan probe targeting PLAC4 rs8130833 SNP
tcgtcgtctaacttg

SEQ ID NO: 16 - DNA, 17 bp, synthetic construct
  source 1..17: mol_type = other DNA
  modified_base 1: mod_base = OTHER; note = a modified by fluorescent reporter VIC
  modified_base 17: mod_base = OTHER; note = g modified by minor groove binding non-fluorescent quencher (MGBNFQ)
  misc_feature 1..17: note = synthetic allele-A-specific TaqMan probe targeting
attcgtcatctaacttg

SEQ ID NO: 17 - DNA, 20 bp, synthetic construct
  source 1..20: mol_type = other DNA
  misc_feature 1..20: note = synthetic digital PCR amplification serpin peptidase inhibitor clade B (ovalbumin) member 2 (SERPINB2) gene-specific reverse transcription primer
cgcagacttctcaccaaaca

SEQ ID NO: 18 - DNA, 20 bp, synthetic construct
  source 1..20: mol_type = other DNA
  misc_feature 1..20: note = synthetic digital PCR amplification serpin peptidase inhibitor clade B (ovalbumin) member 2 (SERPINB2) forward primer
ctcagctctgcaatcaatgc

SEQ ID NO: 19 - DNA, 16 bp, synthetic construct
  source 1..16: mol_type = other DNA
  modified_base 1: mod_base = OTHER; note = c modified by 6-carboxyfluorescein (FAM)
  modified_base 16: mod_base = OTHER; note = t modified by minor groove binding non-fluorescent quencher (MGBNFQ)
  misc_feature 1..16: note = synthetic allele-A-specific TaqMan probe targeting serpin peptidase inhibitor clade B (ovalbumin) member 2 (SERPINB2) rs6098 SNP
ccacagggaattattt

SEQ ID NO: 20 - DNA, 16 bp, synthetic construct
  source 1..16: mol_type = other DNA
  modified_base 1: mod_base = OTHER; note = c modified by 6-carboxyfluorescein (FAM)
  modified_base 16: mod_base = OTHER; note = t modified by minor groove binding non-fluorescent quencher (MGBNFQ)
  misc_feature 1..16: note = synthetic allele-G-specific TaqMan probe targeting serpin peptidase inhibitor clade B (ovalbumin) member 2 (SERPINB2) rs6098 SNP
ccacaggggattattt

SEQ ID NO: 21 - DNA, 23 bp, synthetic construct
  source 1..23: mol_type = other DNA
  misc_feature 1..23: note = synthetic digital PCR analysis co-amplification forward primer for 101-bp amplicon for paralogous loci on chromosome 21 and 1
gttgttctgcaaaaaaccttcga

SEQ ID NO: 22 - DNA, 28 bp, synthetic construct
  source 1..28: mol_type = other DNA
  misc_feature 1..28: note = synthetic digital PCR analysis co-amplification reverse primer for 101-bp amplicon for paralogous loci on chromosome 21 and 1
cttggccagaaatacttcattaccatat

SEQ ID NO: 23 - DNA, 19 bp, synthetic construct
  source 1..19: mol_type = other DNA
  modified_base 1: mod_base = OTHER; note = t modified by 6-carboxyfluorescein (FAM)
  modified_base 19: mod_base = OTHER; note = a modified by minor groove binding non-fluorescent quencher (MGBNFQ)
  misc_feature 1..19: note = synthetic chromosome-specific TaqMan probe designed to target chromosome 21 paralog
tacctccataatgagtaaa

SEQ ID NO: 24 - DNA, 20 bp, synthetic construct
  source 1..20: mol_type = other DNA
  misc_feature 1..20: note = synthetic chromosome-specific TaqMan probe designed to target chromosome 1 paralog
  modified_base 1: mod_base = OTHER; note = c modified by fluorescent reporter VIC
  modified_base 20: mod_base = OTHER; note = a modified by minor groove binding non-fluorescent quencher (MGBNFQ)
cgtacctctgtaatgtgtaa

SEQ ID NO: 25 - DNA, 24 bp, synthetic construct
  source 1..24: mol_type = other DNA
  misc_feature 1..24: note = synthetic digital RCD analysis co-amplification forward primer for 128-bp amplicon for paralogous loci on chromosome 21 and 18
gtacagaaaccacaaactgatcgg

SEQ ID NO: 26 - DNA, 17 bp, synthetic construct
  source 1..17: mol_type = other DNA
  misc_feature 1..17: note = synthetic digital RCD analysis co-amplification reverse primer for 128-bp amplicon for paralogous loci on chromosome 21 and 18
gtccaggctgtgggcct

SEQ ID NO: 27 - DNA, 14 bp, synthetic construct
  source 1..14: mol_type = other DNA
  modified_base 1: mod_base = OTHER; note = a modified by 6-carboxyfluorescein (FAM)
  modified_base 14: mod_base = OTHER; note = a modified by minor groove binding non-fluorescent quencher (MGBNFQ)
  misc_feature 1..14: note = synthetic chromosome-specific TaqMan probe designed to target chromosome 21 paralog
aagaggcgaggcaa

SEQ ID NO: 28 - DNA, 15 bp, synthetic construct
  source 1..15: mol_type = other DNA
  modified_base 1: mod_base = OTHER; note = a modified by fluorescent reporter VIC
  modified_base 15: mod_base = OTHER; note = c modified by minor groove binding non-fluorescent quencher (MGBNFQ)
  misc_feature 1..15: note = synthetic chromosome-specific TaqMan probe designed to target chromosome 18 paralog
aagaggacaggcaac

SEQ ID NO: 29 - DNA, 33 bp, synthetic construct
  source 1..33: mol_type = other DNA
  misc_feature 1..33: note = synthetic digital PCR analysis co-amplification forward primer for 121-bp amplicon for paralogous loci on chromosome 21 and 1
acgttggatggttgttctgcaaaaaaccttcga

SEQ ID NO: 30 - DNA, 38 bp, synthetic construct
  source 1..38: mol_type = other DNA
  misc_feature 1..38: note = synthetic digital PCR analysis co-amplification reverse primer for 121-bp amplicon for paralogous loci on chromosome 21 and 1
acgttggatgcttggccagaaatacttcattaccatat

SEQ ID NO: 31 - DNA, 21 bp, synthetic construct
  source 1..21: mol_type = other DNA
  misc_feature 1..21: note = synthetic digital PCR analysis co-amplification extension primer for 121-bp amplicon for paralogous loci on chromosome 21 and 1
ctcatcctcacttcgtacctc

SEQ ID NO: 32 - DNA, 34 bp, synthetic construct
  source 1..34: mol_type = other DNA
  misc_feature 1..34: note = synthetic digital RCD analysis co-amplification forward primer for 148-bp amplicon for paralogous loci on chromosome 21 and 18
acgttggatggtacagaaaccacaaactgatcgg

SEQ ID NO: 33 - DNA, 27 bp, synthetic construct
  source 1..27: mol_type = other DNA
  misc_feature 1..27: note = synthetic digital RCD analysis co-amplification reverse primer for 148-bp amplicon for paralogous loci on chromosome 21 and 18
acgttggatggtccaggctgtgggcct

SEQ ID NO: 34 - DNA, 17 bp, synthetic construct
  source 1..17: mol_type = other DNA
  misc_feature 1..17: note = synthetic digital RCD analysis co-amplification extension primer for 148-bp amplicon for paralogous loci on chromosome 21 and 18
acaaaagggggaagagg

SEQ ID NO: 35 - DNA, 35 bp, synthetic construct
  source 1..35: mol_type = other DNA
  misc_feature 1..35: note = synthetic digital RCD analysis co-amplification forward primer for 81 bp amplicon for paralogous loci on chromosome 21 and 1
acgttggatgttgatgaagtctcatctctacttcg

SEQ ID NO: 36 - DNA, 33 bp, synthetic construct
  source 1..33: mol_type = other DNA
  misc_feature 1..33: note = synthetic digital RCD analysis co-amplification reverse primer for 81 bp amplicon for paralogous loci on chromosome 21 and 1
acgttggatgcaataagcttggccagaaatact

SEQ ID NO: 37 - DNA, 37 bp, synthetic construct
  source 1..37: mol_type = other DNA
  misc_feature 1..37: note = synthetic digital RCD analysis co-amplification forward primer for 82 bp amplicon for paralogous loci on chromosome 21 and 7
acgttggatggaatttaagctaaatcagcctgaactg

SEQ ID NO: 38 - DNA, 37 bp, synthetic construct
  source 1..37: mol_type = other DNA
  misc_feature 1..37: note = synthetic digital RCD analysis co-amplification reverse primer for 82 bp amplicon for paralogous loci on chromosome 21 and 7
acgttggatggtttctcatagttcatcgtaggcttat

SEQ ID NO: 39 - DNA, 30 bp, synthetic construct
  source 1..30: mol_type = other DNA
  misc_feature 1..30: note = synthetic digital RCD analysis co-amplification forward primer for 101 bp amplicon for paralogous loci on chromosome 21 and 2
acgttggatgtcaggcagggttctatgcag

SEQ ID NO: 40 - DNA, 30 bp, synthetic construct
  source 1..30: mol_type = other DNA
  misc_feature 1..30: note = synthetic digital RCD analysis co-amplification reverse primer for 101 bp amplicon for paralogous loci on chromosome 21 and 2
acgttggatgaggcggcttcctggctcttg

SEQ ID NO: 41 - DNA, 31 bp, synthetic construct
  source 1..31: mol_type = other DNA
  misc_feature 1..31: note = synthetic digital RCD analysis co-amplification forward primer for 102 bp amplicon for paralogous loci on chromosome 21 and 6
acgttggatggctcgtctcaggctcgtagtt

SEQ ID NO: 42 - DNA, 30 bp, synthetic construct
  source 1..30: mol_type = other DNA
  misc_feature 1..30: note = synthetic digital RCD analysis co-amplification reverse primer for 102 bp amplicon for paralogous loci on chromosome 21 and 6
acgttggatgtttcttcgagcccttcttgg

SEQ ID NO: 43 - DNA, 23 bp, synthetic construct
  source 1..23: mol_type = other DNA
  misc_feature 1..23: note = synthetic extension primer for paralogous sequence mismatches (PSM) on paralogous loci on chromosomes 21 and 1
gtctcatctctacttcgtacctc

SEQ ID NO: 44 - DNA, 19 bp, synthetic construct
  source 1..19: mol_type = other DNA
  misc_feature 1..19: note = synthetic extension primer for paralogous sequence mismatches (PSM) on paralogous loci on chromosomes 21 and 7
ttttacgctgtccccattt

SEQ ID NO: 45 - DNA, 19 bp, synthetic construct
  source 1..19: mol_type = other DNA
  misc_feature 1..19: note = synthetic extension primer for paralogous sequence mismatches (PSM) on paralogous loci on chromosomes 21 and 2
ggtctatgcaggagccgac

SEQ ID NO: 46 - DNA, 25 bp, synthetic construct
  source 1..25: mol_type = other DNA
  misc_feature 1..25: note = synthetic extension primer for paralogous sequence mismatches (PSM) on paralogous loci on chromosomes 21 and 6
tgggcgcgggagcggacttcgctgg

SEQ ID NO: 47 - DNA, 25 bp, synthetic construct
  source 1..25: mol_type = other DNA
  misc_feature 1..25: note = synthetic digital PCR analysis co-amplification forward primer for 87-bp amplicon for zinc finger protein sequences on chromosome X (ZFX) and Y (ZFY)
caagtgctggactcagatgtaactg

SEQ ID NO: 48 - DNA, 28 bp, synthetic construct
  source 1..28: mol_type = other DNA
  misc_feature 1..28: note = synthetic digital PCR analysis co-amplification reverse primer for 87-bp amplicon for zinc finger protein sequences on chromosome X (ZFX) and Y (ZFY)
tgaagtaatgtcagaagctaaaacatca

SEQ ID NO: 49 - DNA, 16 bp, synthetic construct
  source 1..16: mol_type = other DNA
  modified_base 1: mod_base = OTHER; note = t modified by fluorescent reporter VIC
  modified_base 16: mod_base = OTHER; note = a modified by minor groove binding non-fluorescent quencher (MGBNFQ)
  misc_feature 1..16: note = synthetic chromosome-specific TaqMan probe designed to target chromosome X paralog
tctttagcacattgca

SEQ ID NO: 50 - DNA, 17 bp, synthetic construct
  source 1..17: mol_type = other DNA
  modified_base 1: mod_base = OTHER; note = t modified by 6-carboxyfluorescein (FAM)
  modified_base 17: mod_base = OTHER; note = c modified by minor groove binding non-fluorescent quencher (MGBNFQ)
  misc_feature 1..17: note = synthetic chromosome-specific TaqMan probe designed to target chromosome Y paralog
tctttaccacactgcac

SEQ ID NO: 51 - DNA, 19 bp, synthetic construct
  source 1..19: mol_type = other DNA
  misc_feature 1..19: note = synthetic digital PCR co-amplification forward primer for 87-bp amplicon of beta-globin (hemoglobin beta (HBB)) HbE mutation forward primer
gggcaaggtgaacgtggat

SEQ ID NO: 52 - DNA, 29 bp, synthetic construct
  source 1..29: mol_type = other DNA
  misc_feature 1..29: note = synthetic digital PCR co-amplification forward primer for 87-bp amplicon of beta-globin (hemoglobin beta (HBB)) HbE mutation reverse primer
ctattggtctccttaaacctgtcttgtaa

SEQ ID NO: 53 - DNA, 14 bp, synthetic construct
  source 1..14: mol_type = other DNA
  modified_base 1: mod_base = OTHER; note = t modified by fluorescent reporter VIC
  modified_base 14: mod_base = OTHER; note = c modified by minor groove binding non-fluorescent quencher (MGBNFQ)
  misc_feature 1..14: note = synthetic allele-G-specific TaqMan probe targeting beta-globin (hemoglobin beta (HBB)) HbE mutation normal allele
ttggtggtgaggcc

SEQ ID NO: 54 - DNA, 14 bp, synthetic construct
  source 1..14: mol_type = other DNA
  modified_base 1: mod_base = OTHER; note = t modified by 6-carboxyfluorescein (FAM)
  modified_base 14: mod_base = OTHER; note = c modified by minor groove binding non-fluorescent quencher (MGBNFQ)
  misc_feature 1..14: note = synthetic allele-A-specific TaqMan probe targeting beta-globin (hemoglobin beta (HBB)) HbE mutation mutant allele
ttggtggtaaggcc

SEQ ID NO: 55 - DNA, 20 bp, synthetic construct
  source 1..20: mol_type = other DNA
  misc_feature 1..20: note = synthetic digital PCR co-amplification forward primer for 87-bp and 83-bp amplicon of CD41/42 deletion mutation normal and mutant allele
ttttcccacccttaggctgc

SEQ ID NO: 56 - DNA, 23 bp, synthetic construct
  source 1..23: mol_type = other DNA
  misc_feature 1..23: note = synthetic digital PCR co-amplification reverse primer for 87-bp and 83-bp amplicon of CD41/42 deletion mutation normal and mutant allele
acagcatcaggagtggacagatc

SEQ ID NO: 57 - DNA, 19 bp, synthetic construct
  source 1..19: mol_type = other DNA
  modified_base 1: mod_base = OTHER; note = c modified by fluorescent reporter VIC
  modified_base 19: mod_base = OTHER; note = t modified by minor groove binding non-fluorescent quencher (MGBNFQ)
  misc_feature 1..19: note = synthetic allele-specific TaqMan probe targeting CD41/42 deletion mutation normal allele (without deletion)
cagaggttctttgagtcct

SEQ ID NO: 58 - DNA, 15 bp, synthetic construct
  source 1..15: mol_type = other DNA
  modified_base 1: mod_base = OTHER; note = a modified by 6-carboxyfluorescein (FAM)
  modified_base 15: mod_base = OTHER; note = t modified by minor groove binding non-fluorescent quencher (MGBNFQ)
  misc_feature 1..15: note = synthetic allele-specific TaqMan probe targeting CD41/42 deletion mutation mutant allele (with deletion)
agaggttgagtcctt